European Patent Application EP 4 715 039 A1, published March 25, 2026. Title: 一种马克斯克鲁维酵母菌株及其应用. Applicant: 安琪酵母股份有限公司. The sequence listing filed with the application follows.

SEQUENCE LISTING (4 sequences)

SEQ ID NO: 1 - DNA, 755 bp, Kluyveromyces marxianus
  source 1..755: mol_type = genomic DNA
tcttccccccccctttttgtatgcttaagttcagcgggtactcctacctgatttgaggtcaaactttgagagttttggttaaagccgtatgcctcaaggagacaaacaccagcgagtctttataacacctatgagtctctatgacccaagcttaccacgaattggcgcaaacctaagacgtagatgtgcaagagtcgagtccatagacttgacacgcagccctgctcacgcagatggcaacggctagccactttcaagttaacccgagacgagtatcactcactaccaaacccaaaggtttgagagagaaatgacgctcaaacaggcatgccccctggaataccagagggcgcaatgtgcgttcaaagatttgatgattcacgaaaatctgcaattcacaatacatatcgcaattcgctgcgttcttcatcgatgcgagaaccaagagatccgttgttgaaagttttgaatattaaattttatagtataatagtttttcataatacaaaatattgtttgtgtttatgtccactggagagacgagctctccagggaagtagttcatagagaaaaaactccattgtgtttaggatgagaaatagaaaactgatagcagagaatcaagaactggccgcgcaattaagcgcaggccttgttcagacgattcccccagtaatctattcattcataatctttaatgatccttccgcaggttcacctacggaaaccttgtatttttttattctctctataaa

SEQ ID NO: 2 - DNA, 725 bp, Kluyveromyces marxianus
  source 1..725: mol_type = genomic DNA
ccttccgtaggtgaacctgcggaaggatcattaaagattatgaatgaatagattactgggggaatcgtctgaacaaggcctgcgcttaattgcgcggccagttcttgattctctgctatcagttttctatttctcatcctaaacacaatggagttttttctctatgaactacttccctggagagctcgtctctccagtggacataaacacaaacaatattttgtattatgaaaaactattatactataaaatttaatattcaaaactttcaacaacggatctcttggttctcgcatcgatgaagaacgcagcgaattgcgatatgtattgtgaattgcagattttcgtgaatcatcaaatctttgaacgcacattgcgccctctggtattccagggggcatgcctgtttgagcgtcatttctctctcaaacctttgggtttggtagtgagtgatactcgtctcgggttaacttgaaagtggctagccgttgccatctgcgtgagcagggctgcgtgtcaagtctatggactcgactcttgcacatctacgtcttaggtttgcgccaattcgtggtaagcttgggtcatagagactcataggtgttataaagactcgctggtgtttgtctccttgaggcatacggctttaaccaaaactctcaaagtttgacctcaaatcaggtaggagtacccgctgaacttaagcatatcaataagcggaggaa

SEQ ID NO: 3 - DNA, 22 bp, primer
  source 1..22: mol_type = other DNA
ggaagtaaaagtcgtaacaagg

SEQ ID NO: 4 - DNA, 20 bp, primer
  source 1..20: mol_type = other DNA
tcctccgcttattgatatgc